European Patent Application EP 4 434 351 A1, published September 25, 2024. Title: A Feed Composition for Preparing An Animal Model for Steatohepatitis. Applicant: Industry-Academic Cooperation Foundation, Yonsei University. Application KR. The sequence listing filed with the application follows.

SEQUENCE LISTING (18 sequences)

SEQ ID NO: 1 - DNA, 19 bp, synthetic construct
  source 1..19: mol_type = other DNA
gctacgacgtgggctacag

SEQ ID NO: 2 - DNA, 23 bp, synthetic construct
  source 1..23: mol_type = other DNA
ccctcacactcagatcatcttct

SEQ ID NO: 3 - DNA, 23 bp, synthetic construct
  source 1..23: mol_type = other DNA
ttaaaaacctggatcggaaccaa

SEQ ID NO: 4 - DNA, 23 bp, synthetic construct
  source 1..23: mol_type = other DNA
gcattagcttcagatttacgggt

SEQ ID NO: 5 - DNA, 21 bp, synthetic construct
  source 1..21: mol_type = other DNA
taagggtccccaatggtgaga

SEQ ID NO: 6 - DNA, 20 bp, synthetic construct
  source 1..20: mol_type = other DNA
gggtccctcgactcctacat

SEQ ID NO: 7 - DNA, 21 bp, synthetic construct
  source 1..21: mol_type = other DNA
gtcccagacatcagggagtaa

SEQ ID NO: 8 - DNA, 21 bp, synthetic construct
  source 1..21: mol_type = other DNA
tcggatacttcagcgtcagga

SEQ ID NO: 9 - DNA, 19 bp, synthetic construct
  source 1..19: mol_type = other DNA
gcagaccacagcgtatcca

SEQ ID NO: 10 - DNA, 20 bp, synthetic construct
  source 1..20: mol_type = other DNA
aacaggtcggacatcaccag

SEQ ID NO: 11 - DNA, 16 bp, synthetic construct
  source 1..16: mol_type = other DNA
cccaacgccccgaact

SEQ ID NO: 12 - DNA, 23 bp, synthetic construct
  source 1..23: mol_type = other DNA
gcagaagagctgctgctacgtga

SEQ ID NO: 13 - DNA, 21 bp, synthetic construct
  source 1..21: mol_type = other DNA
accgaagtcatagccacactc

SEQ ID NO: 14 - DNA, 20 bp, synthetic construct
  source 1..20: mol_type = other DNA
ctccgttacttggggacacc

SEQ ID NO: 15 - DNA, 22 bp, synthetic construct
  source 1..22: mol_type = other DNA
aaggggataacagccactacaa

SEQ ID NO: 16 - DNA, 24 bp, synthetic construct
  source 1..24: mol_type = other DNA
accaacataaaaattaagccaaat

SEQ ID NO: 17 - DNA, 20 bp, synthetic construct
  source 1..20: mol_type = other DNA
cttccagctaccatcccaaa

SEQ ID NO: 18 - DNA, 20 bp, synthetic construct
  source 1..20: mol_type = other DNA
cttcagaggcaggaaacagg